European Patent Specification EP 4 022 095 B1, published August 27, 2025. Title: Detection of Mycobacterium species. Applicant: The Queen's University of Belfast The Queen's University of Belfast. The sequence listing filed with the application follows.

SEQUENCE LISTING (6 sequences)

SEQ ID NO: 1 - DNA, 19 bp, Unknown
  synthetic
ccggtaaggccgaccatta

SEQ ID NO: 2 - DNA, 16 bp, Unknown
  Synthetic
acccgctgcgagagca

SEQ ID NO: 3 - DNA, 26 bp, Unknown
  Synthetic
catggttattaacgacgacgcgcagc

SEQ ID NO: 4 - DNA, 21 bp, Unknown
  Synthetic
aactaagcggatcgacaattc

SEQ ID NO: 5 - DNA, 20 bp, Unknown
  Synthetic
tggtgtaccgaatgttgttg

SEQ ID NO: 6 - DNA, 22 bp, Unknown
  Synthetic
tgcaactcgaacacacctggga